European Patent Application EP 4 321 621 A1, published February 14, 2024. Title: Antibodies to pancreatic cancer stem cells. Applicant: University Public Corporation Osaka Kobe University. The sequence listing filed with the application follows.

SEQUENCE LISTING (30 sequences)

SEQ ID NO: 1 - protein, 115 aa, human
QVQLKESGPGLVQPSQTLSLTCTVSGFSLSSYGVIWVRQPPGKGLEWMGLIWDNGNTNYNSALKSRLSISRDTSKSQVFLKMNNLQTEDTAMYFCARSRHYFDYWGQGVMVTVSS

SEQ ID NO: 2 - protein, 106 aa, human
DIQMTQSPSLLSASVGDRVTLNCKASQNIYKILAWYQQKLGEAPKLLIYNADSLQTGIPSRFSGSGSGTDFTLTISSLQPEDVATYFCQQYYSGWTFGGGTKLELK

SEQ ID NO: 3 - protein, 115 aa, human
QVQLKESGPGLVQPSQTLSLTCTVSGFSLSSYGVIWVRQPPGKGLEWMGLIWDNGDTNYCSPLKSRLSISRDTSKSQVFLKMNNLQTEDTAMYFCARSRHYFDYWGQGVMVTVSS

SEQ ID NO: 4 - protein, 106 aa, human
DIQMTQSPSLLSASVGDRVTLNCKASQNIYKNLAWYQQKLGEAPKFLIYNANSLQTGIPSRFSGSGSGTDFTLTISSLQPEDVATYFCQQYYSGWTFGGGTKLELK

SEQ ID NO: 5 - protein, 122 aa, human
QVQLQQSGAELVKPGSSVKISCKASGYTFTSNFMHWIKQQPGNGLEWIGWISPGDGDTEYNQKFNGKATLTADKSSSTAYMQLSSLTSEDSAVYFCARGGYYSGGGGYFDYWGQGVMVTVSS

SEQ ID NO: 6 - protein, 108 aa, human
DIVMTQSPTSMSISVGDRVTMNCKASQNLGSYVDWYQQKTGQSPKLLIYKASNRYTGVPDRFTGSGSGTDFTFSISNMQAEDLAVYYCMQSNSYLMYTFGAGTKLELK

SEQ ID NO: 7 - protein, 123 aa, human
EVQLVESGGGLVQPGRSLKLSCAASGFTFSDYNMAWVRQAPKKGLEWVATINYDGISTYYRDSVKGRFTISRDNAKSTLYLQMDSLRSEDTATYYCARHSYVYYALGVPFAYWGQGTLVTVSS

SEQ ID NO: 8 - protein, 107 aa, human
DIQMTQSPSLLSASVGDRVTINCKASQNINKYLNWYQQKLGEAPKLLIYNTNSLQTGIPSRFSGSGSGTDYTLTISSLQPEDFGTYFCFQHNSWPLTFGSGTKLEIK

SEQ ID NO: 9 - DNA, 346 bp, human
caggtgcagctgaaggagtcaggacctggcctggtgcagccctcacagaccctgtctctcacctgcactgtctctgggttctcactaagcagctatggtgtaatctgggttcgccagcctccaggaaagggtctggagtggatgggactaatatgggataatggaaatacaaattataattcagctctcaaatcccgactgagcatcagcagggacacctccaagagccaagttttcttaaaaatgaacaatctgcaaactgaagacacagccatgtacttctgtgccagatcgaggcactactttgattactggggccaaggagtcatggtcacagtctcctcag

SEQ ID NO: 10 - DNA, 319 bp, human
gacatccagatgacccagtctccttcactcctgtctgcatctgtgggagacagagtcactctcaactgcaaagcaagtcagaatatttataagatcttagcctggtatcagcaaaagcttggagaagctcccaaactcctgatttataatgcagacagtttgcaaacgggcatcccatcaaggttcagtggcagtggatctggtacagatttcacactcaccatcagcagcctgcagcctgaagatgttgccacatatttctgccagcagtattatagcgggtggacgttcggtggaggcaccaagctggaattgaaac

SEQ ID NO: 11 - DNA, 346 bp, human
caggtgcagctgaaggagtcaggacctggcctggtgcagccctcacagaccctgtctctcacctgcactgtctctgggttctcactaagcagctatggtgtaatctgggttcgccagcctccaggaaagggtctggagtggatgggactaatatgggataatggagatacaaattattgttcacctctcaaatcccgactgagcatcagcagggacacctccaagagccaagttttcttaaaaatgaacaatctgcaaactgaagacacagccatgtacttctgtgccagatcgaggcactactttgattactggggccaaggagtcatggtcacagtctcctcag

SEQ ID NO: 12 - DNA, 319 bp, human
gacatccagatgacccagtctccttcactcctgtctgcatctgtgggagacagagtcactctcaactgcaaagcaagtcagaatatttataagaacttagcctggtatcagcaaaagcttggagaagctcccaaattcctgatttataatgcaaacagtttgcaaacgggcatcccatcaaggttcagtggcagtggatctggtacagatttcacactcaccatcagcagcctgcagcctgaagatgttgccacatatttctgccagcagtattatagcgggtggacgttcggtggaggcaccaagctggaattgaaac

SEQ ID NO: 13 - DNA, 367 bp, human
caggtacagctgcagcaatctggggctgaactggtgaagcctgggtcgtcagtgaaaatttcctgcaaggcttctggctacaccttcaccagtaactttatgcactggataaaacagcagcctggaaatggccttgagtggattgggtggatttctcctggagatggtgatacagagtacaatcaaaagttcaatgggaaggcaacactcactgcagacaaatcctccagcacagcctatatgcagctcagcagcctgacatctgaggactctgcagtctatttctgtgcaagaggggggtactacagtggtggagggggctactttgattactggggccaaggagtcatggtcacagtctcctcag

SEQ ID NO: 14 - DNA, 325 bp, human
gacattgtgatgactcagtctcccacatccatgtccatatcagtaggagacagggtcaccatgaactgcaaggccagtcaaaatttgggttcttatgtagactggtaccaacagaaaacagggcagtctcctaaactgcttatctacaaagcatccaaccggtacacgggagtccctgatcgcttcacaggcagtggatctggaacagatttcactttctccatcagcaacatgcaggctgaagacctggctgtttattactgtatgcagtctaactcctatctcatgtacacgtttggagctgggaccaagctggaactgaaac

SEQ ID NO: 15 - DNA, 370 bp, human
gaggtgcagctggtggagtctgggggaggcttagtgcagcctggaaggtccctgaaactctcctgtgcagcctcaggattcactttcagtgactataacatggcctgggtccgccaggctccaaagaagggtctggagtgggtcgcaaccattaattatgatggtattagcacttactatcgagactccgtgaagggccgattcaccatctccagagataatgcaaaaagcaccctatacctgcaaatggacagcctgaggtctgaggacacggccacttattactgtgctagacattcttatgtatactacgcattaggagtcccgtttgcttactggggccaaggcactctggtcactgtctcttcag

SEQ ID NO: 16 - DNA, 322 bp, human
gacatccagatgacccagtctccttcactcctgtctgcatctgtgggagacagagtcactatcaactgcaaagcaagtcagaatattaacaagtacttaaactggtatcagcaaaagcttggagaagctcccaaactcctgatatataatacaaacagtttgcaaacgggcatcccatcaaggttcagtggcagtggatctggtacagattacacactcaccatcagcagcctgcagcctgaagattttggcacatatttctgctttcagcataatagttggccgctcacgttcggttctgggaccaagctggagatcaaac

SEQ ID NO: 17 - protein, 19 aa, human
MAVLVLLLCLVTLPSCALS

SEQ ID NO: 18 - DNA, 57 bp, human
atggctgtcctagtgctgctcctctgcctggtgacacttccaagctgtgccctgtcc

SEQ ID NO: 19 - protein, 19 aa, human
MAPVQLLGLLVLFLPAMRC

SEQ ID NO: 20 - DNA, 57 bp, human
atggctccagttcaacttttagggcttttggtgctcttcctcccagccatgagatgt

SEQ ID NO: 21 - protein, 19 aa, human
MAVLVLFLCLVTLPSCALS

SEQ ID NO: 22 - DNA, 57 bp, human
atggctgtcttagtgctgttcctctgcctggtgacacttccaagctgtgccctgtcc

SEQ ID NO: 23 - protein, 17 aa, human
MKLPVRLLVLFLPAMRC

SEQ ID NO: 24 - DNA, 51 bp, human
atgaagttgcctgttaggctgttggtgctcttcctcccagccatgagatgt

SEQ ID NO: 25 - protein, 19 aa, human
MGWSCIMFFLVAAATCVHS

SEQ ID NO: 26 - protein, 57 aa, human
ATGGGATGGAGCTGTATCATGTTCTTTCTGGTGGCAGCAGCTACATGTGTTCACTCC

SEQ ID NO: 27 - protein, 20 aa, human
MESQTQVFIFLLLWLSGADG

SEQ ID NO: 28 - DNA, 60 bp, human
atggagtcacagacccaggtcttcatattcctgctgctctggttgtctggtgctgatggg

SEQ ID NO: 29 - protein, 19 aa, human
MDSRLNLVFLVLFMKGVQC

SEQ ID NO: 30 - DNA, 57 bp, human
atggactccaggctcaatttagttttccttgtcctttttatgaaaggtgtccagtgt